European Patent Specification EP 3 094 320 B1, published June 14, 2023. Title: METHODS OF USING CAPSAICIN SYNTHASE FOR THE MICROBIAL PRODUCTION OF CAPSAICINOIDS. Applicant: Conagen, Inc. Application PCT/US. The sequence listing filed with the application follows.

SEQUENCE LISTING (7 sequences)

SEQ ID NO: 1 - DNA, 1323 bp, Ghost Chili Pepper
atggcttttgcattaccatcatcacttgtttcagtttgtgacaaatcttttatcaaaccttcctctctcaccccctctaaacttagatttcacaagctatctttcatcgatcaatctttaagtaatatgtatatcccttgtgcatttttttaccctaaagtacaacaaagactagaagactccaaaaattctgatgagctttcccatatagcccacttgctacaaacatctctatcacaaactctagtctcttactatccttatgcaggaaagttgaaggacaatgctactgttgactgtaacgatatgggagctgagttcttgagtgttcgaataaaatgttccatgtctgaaattcttgatcatcctcatgcatctcttgcagagagcatagttttgcccaaggatttgccttgggcgaataattgtgaaggtggtaatttgcttgtagttcaagtaagtaagtttgattgtgggggaatagccatcagtgtatgcttttcgcacaagattggtgatggttgctctctgcttaatttccttaatgattggtctagcgttactcgtgatcatacgacaacagctttagttccatctcctagatttgtaggagattctgtcttctctacaaaaaaatatggttctcttattacgccacaaattttgtccgatctcaacgagtgcgtacagaaaagactcatttttcctacagataagttagatgcacttcgagctaaggtggcagaagaatcaggagtaaaaaatccaacaagggcagaagttgttagcgctcttcttttcaaatgtgcaacaaaggcatcatcatcaatgctaccatcaaagttggttcacttcttaaacatacgtactatgatcaaacctcgtctaccacgaaatgccattggaaatctctcgtctattttctccatagaagcaactaacatgcaggacatggagttgccaacgttggttcgtaatttaaggaaggaagttgaggtggcatacaagaaagaccaagtcgaacaaaatgaactgatcctagaagtagtagaatcaatgagagaagggaaactgccatttgaaaatatggatggctatgagaatgtgtatacttgcagcaatctttgcaaatatccgtactacactgtagattttggatggggaagacctgaaagagtgtgtctaggaaatggtccctccaagaatgccttcttcttgaaagattacaaagctgggcaaggcgtggaggcgcgggtgatgttgcacaagcaacaaatgtctgaatttgaacgcaatgaggaactccttgagttcattgcctaa

SEQ ID NO: 2 - DNA, 24 bp, Artificial Sequence
  One of the primers for the initial cloning of CS/AT3/Pun1 gene was into the pENTR/D_TOPO vector
caccatggcttttgcattaccatc

SEQ ID NO: 3 - DNA, 21 bp, Artificial Sequence
  One of the primers for the initial cloning of CS/AT3/Pun1 gene into the pENTR/D_TOPO vector
ttaggcaatgaactcaaggag

SEQ ID NO: 4 - DNA, 35 bp, Artificial Sequence
  Primers for cloning CS/Pun1/AT3 gene into pETite N-His SUMO Kan expression vector.
cgcgaacagattggaggtgcttttgcattaccatc

SEQ ID NO: 5 - DNA, 39 bp, Artificial Sequence
  Primer for cloning CS/Pun1/AT3 gene into pETite N-His SUMO Kan expression vector.
gtggcggccgctctattattaggcaatgaactcaaggag

SEQ ID NO: 6 - DNA, 27 bp, Artificial Sequence
  One of the primers for the cloning of ACS1 into pCDFDuet-1 vector.
gaagatctatggcaacagataaattta

SEQ ID NO: 7 - DNA, 28 bp, Artificial Sequence
  One of the primers for the cloning of ACS1 into pCDFDuet-1 vector.
ccgctcgagtcacttggtacccttgtac